European Patent Application EP 4 652 926 A2, published November 26, 2025. Title: ANTI-C1S ANTIBODIES AND METHODS OF USE THEREOF. Applicant: Bioverative USA, Inc. Application EP, filed October 12, 2017. The sequence listing filed with the application follows.

SEQUENCE LISTING (54 sequences)

SEQ ID NO: 1 - protein, 15 aa, synthetic construct
  REGION 1..15: note = VL CDR1
KASQSVDYDGDSYMN

SEQ ID NO: 2 - protein, 7 aa, synthetic construct
  REGION 1..7: note = VL CDR2
DASNLES

SEQ ID NO: 3 - protein, 9 aa, synthetic construct
  REGION 1..9: note = VL CDR3
QQSNEDPWT

SEQ ID NO: 4 - protein, 5 aa, synthetic construct
  REGION 1..5: note = VH CDR1
DDYIH

SEQ ID NO: 5 - protein, 17 aa, synthetic construct
  REGION 1..17: note = VH CDR2
RIDPADGHTKYAPKFQV

SEQ ID NO: 6 - protein, 10 aa, synthetic construct
  REGION 1..10: note = VH CDR3
YGYGREVFDY

SEQ ID NO: 7 - protein, 111 aa, synthetic construct
  REGION 1..111: note = Parental Murine anti-C1s VL Variable Light
DIVLTQSPASLAVSLGQRATISCKASQSVDYDGDSYMNWYQQKTGQPPKILIYDASNLESGIPARFSGSGSGTDFTLNIHPVEEEDAAIYYCQQSNEDPWTFGGGTKLEIK

SEQ ID NO: 8 - protein, 119 aa, synthetic construct
  REGION 1..119: note = VH CDR of an anti-C1s antibody
EVQLQQSGAELVRPGASVKLSCTASGFNIKDDYIHWVKQRPEQGLEWIGRIDPADGHTKYAPKFQVKATITADTSSNTAYLQLSSLTSEDTAVYYCARYGYGREVFDYWGQGTTLTVSS

SEQ ID NO: 9 - protein, 673 aa, synthetic construct
  REGION 1..673: note = Human C1s
EPTMYGEILSPNYPQAYPSEVEKSWDIEVPEGYGIHLYFTHLDIELSENCAYDSVQIISGDTEEGRLCGQRSSNNPHSPIVEEFQVPYNKLQVIFKSDFSNEERFTGFAAYYVATDINECTDFVDVPCSHFCNNFIGGYFCSCPPEYFLHDDMKNCGVNCSGDVFTALIGEIASPNYPKPYPENSRCEYQIRLEKGFQVVVTLRREDFDVEAADSAGNCLDSLVFVAGDRQFGPYCGHGFPGPLNIETKSNALDIIFQTDLTGQKKGWKLRYHGDPMPCPKEDTPNSVWEPAKAKYVFRDVVQITCLDGFEVVEGRVGATSFYSTCQSNGKWSNSKLKCQPVDCGIPESIENGKVEDPESTLFGSVIRYTCEEPYYYMENGGGGEYHCAGNGSWVNEVLGPELPKCVPVCGVPREPFEEKQRIIGGSDADIKNFPWQVFFDNPWAGGALINEYWVLTAAHVVEGNREPTMYVGSTSVQTSRLAKSKMLTPEHVFIHPGWKLLEVPEGRTNFDNDIALVRLKDPVKMGPTVSPICLPGTSSDYNLMDGDLGLISGWGRTEKRDRAVRLKAARLPVAPLRKCKEVKVEKPTADAEAYVFTPNMICAGGEKGMDSCKGDSGGAFAVQDPNDKTKFYAAGLVSWGPQCGTYGLYTRVKNYVDWIMKTMQENSTPRED

SEQ ID NO: 10 - protein, 119 aa, synthetic construct
  REGION 1..119: note = VH1 Variant
EVQLVQSGAELKKPGASVKLSCTASGFNIKDDYIHWVKQAPGQGLEWIGRIDPADGHTKYAPKFQVKATITADTSTNTAYLQLSSLTSEDTAVYYCARYGYGREVFDYWGQGTTVTVSS

SEQ ID NO: 11 - DNA, 357 bp, synthetic construct
  misc_feature 1..357: note = VH variant 1
  source 1..357: mol_type = other DNA
gaggttcagctggtgcagtctggggctgagcttaagaagccaggggcctcagtcaagttgtcctgcacagcttctggctttaacattaaagacgactatatacactgggtgaagcaggcccctggacagggcctggagtggattggaaggattgatcctgcggatggtcatactaaatatgccccgaagttccaagtcaaggccactataactgcagacacatccaccaacacagcctacctgcagctcagcagcctgacatctgaggacactgccgtctattactgtgctagatatggttacgggagggaggtctttgactactggggccaaggcaccactgtcacagtctcctca

SEQ ID NO: 12 - protein, 119 aa, synthetic construct
  REGION 1..119: note = VH2 variant
EVQLVQSGAEVKKPGASVKLSCTASGFNIKDDYIHWVKQAPGQGLEWIGRIDPADGHTKYAPKFQVKATITADTSTNTAYLELSSLRSEDTAVYYCARYGYGREVFDYWGQGTTVTVSS

SEQ ID NO: 13 - DNA, 357 bp, synthetic construct
  misc_feature 1..357: note = VH variant 2
  source 1..357: mol_type = other DNA
gaggttcagctggtgcagtctggggctgaggtgaagaagccaggggcctcagtcaagttgtcctgcacagcttctggctttaacattaaagacgactatatacactgggtgaagcaggcccctggacagggcctggagtggattggaaggattgatcctgcggatggtcatactaaatatgccccgaagttccaagtcaaggccactataactgcagacacatccaccaacacagcctacctggagctcagcagcctgagatctgaggacactgccgtctattactgtgctagatatggttacgggagggaggtctttgactactggggccaaggcaccactgtcacagtctcctca

SEQ ID NO: 14 - protein, 119 aa, synthetic construct
  REGION 1..119: note = VH3 variant
QVQLVQSGAEVKKPGASVKLSCTASGFNIKDDYIHWVKQAPGQGLEWIGRIDPADGHTKYAPKFQVKVTITADTSTSTAYLELSSLRSEDTAVYYCARYGYGREVFDYWGQGTTVTVSS

SEQ ID NO: 15 - DNA, 357 bp, synthetic construct
  misc_feature 1..357: note = VH variant 3
  source 1..357: mol_type = other DNA
caggttcagctggtgcagtctggggctgaggtgaagaagccaggggcctcagtcaagttgtcctgcacagcttctggctttaacattaaagacgactatatacactgggtgaagcaggcccctggacagggcctggagtggattggaaggattgatcctgcggatggtcatactaaatatgccccgaagttccaagtcaaagtcactataactgcagacacatccaccagcacagcctacctggagctcagcagcctgagatctgaggacactgccgtctattactgtgctagatatggttacgggagggaggtctttgactactggggccaaggcaccactgtcacagtctcctca

SEQ ID NO: 16 - protein, 119 aa, synthetic construct
  REGION 1..119: note = VH4 variant
QVQLVQSGAEVKKPGASVKVSCTASGFNIKDDYIHWVRQAPGQGLEWIGRIDPADGHTKYAPKFQVKVTITADTSTSTAYMELSSLRSEDTAVYYCARYGYGREVFDYWGQGTTVTVSS

SEQ ID NO: 17 - DNA, 357 bp, synthetic construct
  misc_feature 1..357: note = VH variant 4
  source 1..357: mol_type = other DNA
caggttcagctggtgcagtctggggctgaggtgaagaagccaggggcctcagtcaaggtctcctgcacagcttctggctttaacattaaagacgactatatacactgggtgcgccaggcccctggacagggcctggagtggattggaaggattgatcctgcggatggtcatactaaatatgccccgaagttccaagtcaaagtcactataactgcagacacatccaccagcacagcctacatggagctcagcagcctgagatctgaggacactgccgtctattactgtgctagatatggttacgggagggaggtctttgactactggggccaaggcaccactgtcacagtctcctca

SEQ ID NO: 18 - protein, 119 aa, synthetic construct
  REGION 1..119: note = VH5 variant
QVQLVQSGAEVKKPGASVKVSCAASGFNIKDDYIHWVRQAPGQGLEWIGRIDPADGHTKYAPKFQVKVTITADTSTSTAYMELSSLRSEDTAVYYCARYGYGREVFDYWGQGTTVTVSS

SEQ ID NO: 19 - DNA, 357 bp, synthetic construct
  misc_feature 1..357: note = VH variant 5
  source 1..357: mol_type = other DNA
caggttcagctggtgcagtctggggctgaggtgaagaagccaggggcctcagtcaaggtctcctgcgcagcttctggctttaacattaaagacgactatatacactgggtgcgccaggcccctggacagggcctggagtggattggaaggattgatcctgcggatggtcatactaaatatgccccgaagttccaagtcaaagtcactataactgcagacacatccaccagcacagcctacatggagctcagcagcctgagatctgaggacactgccgtctattactgtgctagatatggttacgggagggaggtctttgactactggggccaaggcaccactgtcacagtctcctca

SEQ ID NO: 20 - protein, 111 aa, synthetic construct
  REGION 1..111: note = Vkappa1 variant Variable Light
DIVLTQSPDSLAVSLGERATISCKASQSVDYDGDSYMNWYQQKTGQPPKILIYDASNLESGIPARFSGSGSGTDFTLTISSLEEEDFAIYYCQQSNEDPWTFGGGTKVEIK

SEQ ID NO: 21 - DNA, 333 bp, synthetic construct
  misc_feature 1..333: note = Vkappa variant 1
  source 1..333: mol_type = other DNA
gacattgtgctgacccaatctccagactctttggctgtgtctctcggggagagggccaccatctcctgcaaggccagccaaagtgttgattatgatggtgatagttatatgaactggtaccaacaaaaaacaggacagccacccaaaatcctcatttatgatgcatccaatttggaatctggcatcccagccaggtttagtggcagtgggtctgggacagacttcaccctcaccatcagcagcctggaggaggaggattttgcaatctattactgtcagcaaagtaatgaagacccgtggacgttcggtggaggcaccaaggtggaaatcaaa

SEQ ID NO: 22 - protein, 111 aa, synthetic construct
  REGION 1..111: note = Vkappa2 variant Variable Light
DIVLTQSPDSLAVSLGERATISCKASQSVDYDGDSYMNWYQQKPGQPPKILIYDASNLESGIPARFSGSGSGTDFTLTISSLEPEDFAIYYCQQSNEDPWTFGGGTKVEIK

SEQ ID NO: 23 - DNA, 333 bp, synthetic construct
  misc_feature 1..333: note = Vkappa variant 2
  source 1..333: mol_type = other DNA
gacattgtgctgacccaatctccagactctttggctgtgtctctcggggagagggccaccatctcctgcaaggccagccaaagtgttgattatgatggtgatagttatatgaactggtaccaacaaaaaccaggacagccacccaaaatcctcatttatgatgcatccaatttggaatctggcatcccagccaggtttagtggcagtgggtctgggacagacttcaccctcaccatcagcagcctggagcctgaggattttgcaatctattactgtcagcaaagtaatgaagacccgtggacgttcggtggaggcaccaaggtggaaatcaaa

SEQ ID NO: 24 - protein, 111 aa, synthetic construct
  REGION 1..111: note = Vkappa5 variant Variable Light
DIVLTQSPDSLAVSLGERATISCKASQSVDYDGDSYMNWYQQKPGQPPKLLIYDASNLESGIPARFSGSGSGTDFTLTISSLEPEDFAVYYCQQSNEDPWTFGGGTKVEIK

SEQ ID NO: 25 - DNA, 333 bp, synthetic construct
  misc_feature 1..333: note = Vkappa variant 5
  source 1..333: mol_type = other DNA
gacattgtgctgacccaatctccagactctttggctgtgtctctcggggagagggccaccatctcctgcaaggccagccaaagtgttgattatgatggtgatagttatatgaactggtaccaacaaaaaccaggacagccacccaaactcctcatttatgatgcatccaatttggaatctggcatcccagccaggtttagtggcagtgggtctgggacagacttcaccctcaccatcagcagcctggagcctgaggattttgcagtctattactgtcagcaaagtaatgaagacccgtggacgttcggtggaggcaccaaggtggaaatcaaa

SEQ ID NO: 26 - protein, 119 aa, synthetic construct
  REGION 1..119: note = VH region of anti-C1s antibody
  SITE 1: note = MISC_FEATURE - may be Gln or Glu
  SITE 5: note = MISC_FEATURE - may be Val or Gln
  SITE 11: note = MISC_FEATURE - may be Val or Leu
  SITE 20: note = MISC_FEATURE - may be Leu or Val
  SITE 23: note = MISC_FEATURE - may be Thr or Ala
  SITE 38: note = MISC_FEATURE - may be Lys or Arg
  SITE 68: note = MISC_FEATURE - may be Val or Ala
  SITE 77: note = MISC_FEATURE - may be Ser or Asn
  SITE 81: note = MISC_FEATURE - may be Leu or Met
  SITE 82: note = MISC_FEATURE - may be Glu or Gln
  SITE 87: note = MISC_FEATURE - may be Arg or Thr
XVQLXQSGAEXKKPGASVKXSCXASGFNIKDDYIHWVXQAPGQGLEWIGRIDPADGHTKYAPKFQVKXTITADTSTXTAYXXLSSLXSEDTAVYYCARYGYGREVFDYWGQGTTVTVSS

SEQ ID NO: 27 - protein, 111 aa, synthetic construct
  REGION 1..111: note = VL region of anti-C1s antibody
  SITE 44: note = MISC_FEATURE - may be Thr or Pro
  SITE 50: note = MISC_FEATURE - may be Ile or Leu
  SITE 84: note = MISC_FEATURE - may be Glu or Pro
  SITE 89: note = MISC_FEATURE - may be Ile or Val
DIVLTQSPDSLAVSLGERATISCKASQSVDYDGDSYMNWYQQKXGQPPKXLIYDASNLESGIPARFSGSGSGTDFTLTISSLEXEDFAXYYCQQSNEDPWTFGGGTKVEIK

SEQ ID NO: 28 - protein, 327 aa, synthetic construct
  REGION 1..327: note = Human IgG4 Constant Region (Fc) Variant 2
ASTKGPSVFPLAPCSRSTSESTAALGCLVKDYFPEPVTVSWNSGALTSGVHTFPAVLQSSGLYSLSSVVTVPSSSLGTKTYTCNVDHKPSNTKVDKRVESKYGPPCPPCPAPEFEGGPSVFLFPPKPKDTLMISRTPEVTCVVVDVSQEDPEVQFNWYVDGVEVHNAKTKPREEQFNSTYRVVSVLTVLHQDWLNGKEYKCKVSNKGLPSSIEKTISKAKGQPREPQVYTLPPSQEEMTKNQVSLTCLVKGFYPSDIAVEWESNGQPENNYKTTPPVLDSDGSFFLYSRLTVDKSRWQEGNVFSCSVLHEALHSHYTQKSLSLSLGK

SEQ ID NO: 29 - protein, 446 aa, synthetic construct
  REGION 1..446: note = VH3 Mature Heavy Chain
QVQLVQSGAEVKKPGASVKLSCTASGFNIKDDYIHWVKQAPGQGLEWIGRIDPADGHTKYAPKFQVKVTITADTSTSTAYLELSSLRSEDTAVYYCARYGYGREVFDYWGQGTTVTVSSASTKGPSVFPLAPCSRSTSESTAALGCLVKDYFPEPVTVSWNSGALTSGVHTFPAVLQSSGLYSLSSVVTVPSSSLGTKTYTCNVDHKPSNTKVDKRVESKYGPPCPPCPAPEFEGGPSVFLFPPKPKDTLMISRTPEVTCVVVDVSQEDPEVQFNWYVDGVEVHNAKTKPREEQFNSTYRVVSVLTVLHQDWLNGKEYKCKVSNKGLPSSIEKTISKAKGQPREPQVYTLPPSQEEMTKNQVSLTCLVKGFYPSDIAVEWESNGQPENNYKTTPPVLDSDGSFFLYSRLTVDKSRWQEGNVFSCSVLHEALHSHYTQKSLSLSLGK

SEQ ID NO: 30 - protein, 218 aa, synthetic construct
  REGION 1..218: note = Vkappa2 variant Mature Light Chain
DIVLTQSPDSLAVSLGERATISCKASQSVDYDGDSYMNWYQQKPGQPPKILIYDASNLESGIPARFSGSGSGTDFTLTISSLEPEDFAIYYCQQSNEDPWTFGGGTKVEIKRTVAAPSVFIFPPSDEQLKSGTASVVCLLNNFYPREAKVQWKVDNALQSGNSQESVTEQDSKDSTYSLSSTLTLSKADYEKHKVYACEVTHQGLSSPVTKSFNRGEC

SEQ ID NO: 31 - protein, 465 aa, synthetic construct
  REGION 1..465: note = synthetic amino acid sequence
MGWSLILLFLVAVATRVHSQVQLVQSGAEVKKPGASVKLSCTASGFNIKDDYIHWVKQAPGQGLEWIGRIDPADGHTKYAPKFQVKVTITADTSTSTAYLELSSLRSEDTAVYYCARYGYGREVFDYWGQGTTVTVSSASTKGPSVFPLAPCSRSTSESTAALGCLVKDYFPEPVTVSWNSGALTSGVHTFPAVLQSSGLYSLSSVVTVPSSSLGTKTYTCNVDHKPSNTKVDKRVESKYGPPCPPCPAPEFEGGPSVFLFPPKPKDTLMISRTPEVTCVVVDVSQEDPEVQFNWYVDGVEVHNAKTKPREEQFNSTYRVVSVLTVLHQDWLNGKEYKCKVSNKGLPSSIEKTISKAKGQPREPQVYTLPPSQEEMTKNQVSLTCLVKGFYPSDIAVEWESNGQPENNYKTTPPVLDSDGSFFLYSRLTVDKSRWQEGNVFSCSVLHEALHSHYTQKSLSLSLGK

SEQ ID NO: 32 - protein, 238 aa, synthetic construct
  REGION 1..238: note = synthetic amino acid sequence
MRVPAQLLGLLLLWLPGARCDIVLTQSPDSLAVSLGERATISCKASQSVDYDGDSYMNWYQQKPGQPPKILIYDASNLESGIPARFSGSGSGTDFTLTISSLEPEDFAIYYCQQSNEDPWTFGGGTKVEIKRTVAAPSVFIFPPSDEQLKSGTASVVCLLNNFYPREAKVQWKVDNALQSGNSQESVTEQDSKDSTYSLSSTLTLSKADYEKHKVYACEVTHQGLSSPVTKSFNRGEC

SEQ ID NO: 33 - protein, 11 aa, synthetic construct
  REGION 1..11: note = VL CDR1 (CDR-L1) of anti-C1s antibody
SQSVDYDGDSY

SEQ ID NO: 34 - skipped

SEQ ID NO: 35 - protein, 6 aa, synthetic construct
  REGION 1..6: note = VL CDR3 (CDR-L3) of anti-C1s antibody
SNEDPW

SEQ ID NO: 36 - protein, 7 aa, synthetic construct
  REGION 1..7: note = VH CDR1 (CDR-H1) of anti-C1s antibody
GFNIKDD

SEQ ID NO: 37 - skipped

SEQ ID NO: 38 - protein, 8 aa, synthetic construct
  REGION 1..8: note = VH CDR3 (CDR-H3) of anti-C1s antibody
GYGREVFD

SEQ ID NO: 39 - protein, 7 aa, synthetic construct
  REGION 1..7: note = VL CDR1 (CDR-L1) of anti-C1s antibody
DSYMNWY

SEQ ID NO: 40 - protein, 10 aa, synthetic construct
  REGION 1..10: note = VL CDR2 (CDR-L2) of anti-C1s antibody
ILIYDASNLE

SEQ ID NO: 41 - protein, 8 aa, synthetic construct
  REGION 1..8: note = VL CDR3 (CDR-L3) of anti-C1s antibody
QQSNEDPW

SEQ ID NO: 42 - protein, 6 aa, synthetic construct
  REGION 1..6: note = VH CDR1 (CDR-H1) of anti-C1s antibody
KDDYIH

SEQ ID NO: 43 - protein, 13 aa, synthetic construct
  REGION 1..13: note = VH CDR2 (CDR-H2) of anti-C1s antibody
WIGRIDPADGHTK

SEQ ID NO: 44 - protein, 11 aa, synthetic construct
  REGION 1..11: note = VH CDR3 (CDR-H3) of anti-C1s antibody
ARYGYGREVFD

SEQ ID NO: 45 - protein, 107 aa, synthetic construct [sequence omitted]

SEQ ID NO: 46 - protein, 446 aa, synthetic construct
  REGION 1..446: note = VH1 Mature Heavy Chain
EVQLVQSGAELKKPGASVKLSCTASGFNIKDDYIHWVKQAPGQGLEWIGRIDPADGHTKYAPKFQVKATITADTSTNTAYLQLSSLTSEDTAVYYCARYGYGREVFDYWGQGTTVTVSSASTKGPSVFPLAPCSRSTSESTAALGCLVKDYFPEPVTVSWNSGALTSGVHTFPAVLQSSGLYSLSSVVTVPSSSLGTKTYTCNVDHKPSNTKVDKRVESKYGPPCPPCPAPEFEGGPSVFLFPPKPKDTLMISRTPEVTCVVVDVSQEDPEVQFNWYVDGVEVHNAKTKPREEQFNSTYRVVSVLTVLHQDWLNGKEYKCKVSNKGLPSSIEKTISKAKGQPREPQVYTLPPSQEEMTKNQVSLTCLVKGFYPSDIAVEWESNGQPENNYKTTPPVLDSDGSFFLYSRLTVDKSRWQEGNVFSCSVLHEALHSHYTQKSLSLSLGK

SEQ ID NO: 47 - protein, 446 aa, synthetic construct
  REGION 1..446: note = VH2 Mature Heavy Chain
EVQLVQSGAEVKKPGASVKLSCTASGFNIKDDYIHWVKQAPGQGLEWIGRIDPADGHTKYAPKFQVKATITADTSTNTAYLELSSLRSEDTAVYYCARYGYGREVFDYWGQGTTVTVSSASTKGPSVFPLAPCSRSTSESTAALGCLVKDYFPEPVTVSWNSGALTSGVHTFPAVLQSSGLYSLSSVVTVPSSSLGTKTYTCNVDHKPSNTKVDKRVESKYGPPCPPCPAPEFEGGPSVFLFPPKPKDTLMISRTPEVTCVVVDVSQEDPEVQFNWYVDGVEVHNAKTKPREEQFNSTYRVVSVLTVLHQDWLNGKEYKCKVSNKGLPSSIEKTISKAKGQPREPQVYTLPPSQEEMTKNQVSLTCLVKGFYPSDIAVEWESNGQPENNYKTTPPVLDSDGSFFLYSRLTVDKSRWQEGNVFSCSVLHEALHSHYTQKSLSLSLGK

SEQ ID NO: 48 - protein, 446 aa, synthetic construct
  REGION 1..446: note = VH4 Mature Heavy Chain
QVQLVQSGAEVKKPGASVKVSCTASGFNIKDDYIHWVRQAPGQGLEWIGRIDPADGHTKYAPKFQVKVTITADTSTSTAYMELSSLRSEDTAVYYCARYGYGREVFDYWGQGTTVTVSSASTKGPSVFPLAPCSRSTSESTAALGCLVKDYFPEPVTVSWNSGALTSGVHTFPAVLQSSGLYSLSSVVTVPSSSLGTKTYTCNVDHKPSNTKVDKRVESKYGPPCPPCPAPEFEGGPSVFLFPPKPKDTLMISRTPEVTCVVVDVSQEDPEVQFNWYVDGVEVHNAKTKPREEQFNSTYRVVSVLTVLHQDWLNGKEYKCKVSNKGLPSSIEKTISKAKGQPREPQVYTLPPSQEEMTKNQVSLTCLVKGFYPSDIAVEWESNGQPENNYKTTPPVLDSDGSFFLYSRLTVDKSRWQEGNVFSCSVLHEALHSHYTQKSLSLSLGK

SEQ ID NO: 49 - protein, 446 aa, synthetic construct
  REGION 1..446: note = VH5 Mature Heavy Chain
QVQLVQSGAEVKKPGASVKVSCAASGFNIKDDYIHWVRQAPGQGLEWIGRIDPADGHTKYAPKFQVKVTITADTSTSTAYMELSSLRSEDTAVYYCARYGYGREVFDYWGQGTTVTVSSASTKGPSVFPLAPCSRSTSESTAALGCLVKDYFPEPVTVSWNSGALTSGVHTFPAVLQSSGLYSLSSVVTVPSSSLGTKTYTCNVDHKPSNTKVDKRVESKYGPPCPPCPAPEFEGGPSVFLFPPKPKDTLMISRTPEVTCVVVDVSQEDPEVQFNWYVDGVEVHNAKTKPREEQFNSTYRVVSVLTVLHQDWLNGKEYKCKVSNKGLPSSIEKTISKAKGQPREPQVYTLPPSQEEMTKNQVSLTCLVKGFYPSDIAVEWESNGQPENNYKTTPPVLDSDGSFFLYSRLTVDKSRWQEGNVFSCSVLHEALHSHYTQKSLSLSLGK

SEQ ID NO: 50 - protein, 218 aa, synthetic construct
  REGION 1..218: note = Vkappa1 variant Mature Light Chain
DIVLTQSPDSLAVSLGERATISCKASQSVDYDGDSYMNWYQQKTGQPPKILIYDASNLESGIPARFSGSGSGTDFTLTISSLEEEDFAIYYCQQSNEDPWTFGGGTKVEIKRTVAAPSVFIFPPSDEQLKSGTASVVCLLNNFYPREAKVQWKVDNALQSGNSQESVTEQDSKDSTYSLSSTLTLSKADYEKHKVYACEVTHQGLSSPVTKSFNRGEC

SEQ ID NO: 51 - protein, 218 aa, synthetic construct
  REGION 1..218: note = Vkappa5 variant Mature Light Chain
DIVLTQSPDSLAVSLGERATISCKASQSVDYDGDSYMNWYQQKPGQPPKLLIYDASNLESGIPARFSGSGSGTDFTLTISSLEPEDFAVYYCQQSNEDPWTFGGGTKVEIKRTVAAPSVFIFPPSDEQLKSGTASVVCLLNNFYPREAKVQWKVDNALQSGNSQESVTEQDSKDSTYSLSSTLTLSKADYEKHKVYACEVTHQGLSSPVTKSFNRGEC

SEQ ID NO: 52 - protein, 327 aa, synthetic construct
  REGION 1..327: note = Human IgG4 Constant Region (Fc)
ASTKGPSVFPLAPCSRSTSESTAALGCLVKDYFPEPVTVSWNSGALTSGVHTFPAVLQSSGLYSLSSVVTVPSSSLGTKTYTCNVDHKPSNTKVDKRVESKYGPPCPSCPAPEFLGGPSVFLFPPKPKDTLMISRTPEVTCVVVDVSQEDPEVQFNWYVDGVEVHNAKTKPREEQFNSTYRVVSVLTVLHQDWLNGKEYKCKVSNKGLPSSIEKTISKAKGQPREPQVYTLPPSQEEMTKNQVSLTCLVKGFYPSDIAVEWESNGQPENNYKTTPPVLDSDGSFFLYSRLTVDKSRWQEGNVFSCSVMHEALHNHYTQKSLSLSLGK

SEQ ID NO: 53 - protein, 327 aa, synthetic construct
  REGION 1..327: note = Human IgG4 Constant Region (Fc) Variant 1
ASTKGPSVFPLAPCSRSTSESTAALGCLVKDYFPEPVTVSWNSGALTSGVHTFPAVLQSSGLYSLSSVVTVPSSSLGTKTYTCNVDHKPSNTKVDKRVESKYGPPCPPCPAPEFEGGPSVFLFPPKPKDTLMISRTPEVTCVVVDVSQEDPEVQFNWYVDGVEVHNAKTKPREEQFNSTYRVVSVLTVLHQDWLNGKEYKCKVSNKGLPSSIEKTISKAKGQPREPQVYTLPPSQEEMTKNQVSLTCLVKGFYPSDIAVEWESNGQPENNYKTTPPVLDSDGSFFLYSRLTVDKSRWQEGNVFSCSVMHEALHNHYTQKSLSLSLGK

SEQ ID NO: 54 - protein, 218 aa, synthetic construct
  REGION 1..218: note = Parental Murine anti-C1s VL Mature Light Chain
DIVLTQSPASLAVSLGQRATISCKASQSVDYDGDSYMNWYQQKTGQPPKILIYDASNLESGIPARFSGSGSGTDFTLNIHPVEEEDAAIYYCQQSNEDPWTFGGGTKLEIKRTVAAPSVFIFPPSDEQLKSGTASVVCLLNNFYPREAKVQWKVDNALQSGNSQESVTEQDSKDSTYSLSSTLTLSKADYEKHKVYACEVTHQGLSSPVTKSFNRGEC